European Patent Application EP 4 495 116 A1, published January 22, 2025. Title: Nitrogen-containing heterocyclic compound. Applicant: SHANGHAI SHIJIANG BIOTECHNOLOGY CO., LTD. Application EP. The sequence listing filed with the application follows.

SEQUENCE LISTING (1 sequence)

SEQ ID NO: 1 - DNA, 21 bp, synthetic construct
  source 1..21: mol_type = other DNA
gttcttcatctgcaccataaa